European Patent Application EP 4 556 019 A1, published May 21, 2025. Title: ANTIGEN COMPOSITION, COMPOSITION FOR ANTIGEN EXPRESSION, AND ANTIBODY COMPOSITION. Applicant: USHIO DENKI KABUSHIKI KAISHA. Application EP PCT/JP2023/025593, filed July 11, 2023. The sequence listing filed with the application follows.

SEQUENCE LISTING (5 sequences)

SEQ ID NO: 1 - protein, 51 aa, Homo sapiens
MSKRSWWAGSRKPPREMLKLSGSDSSQSMNGLEVAPPGLITNFSLATAEQC

SEQ ID NO: 2 - protein, 5 aa, Homo sapiens
NHWPF

SEQ ID NO: 3 - protein, 15 aa, Homo sapiens
PQTVQTNHTVVCLQL

SEQ ID NO: 4 - skipped

SEQ ID NO: 5 - protein, 36 aa, Homo sapiens
MSKRSWWAGSRKPPREMLKLSGSDSSQSMNGLEVAP